European Patent Application EP 4 253 397 A1, published October 4, 2023. Title: Peptide Having Activity of Protecting Cell Damage From Particulate Matter and Uses Thereof. Applicant: CAREGEN CO., LTD. The sequence listing filed with the application follows.

SEQUENCE LISTING (1 sequence)

SEQ ID NO: 1 - protein, 3 aa, Artificial Sequence
  Artificial Peptide
WYM